European Patent Specification EP 3 788 059 B1, published August 13, 2025. Title: STEVIOL GLYCOSIDE TRANSPORT. Applicant: DSM IP Assets B.V. The sequence listing filed with the application follows.

SEQUENCE LISTING (6 sequences)

SEQ ID NO: 1 - DNA, 4296 bp, Yarrowia lipolytica
  misc_feature: Polynucleotide sequence of the Open Reading Frame (ORF) belonging to the Yarrowia lipolytica transporter YALI0E25201
atgggtaaaaccgaagtgacacaggagagtctagaatgcgggtcggtcacgtcctcgctggggaaaaagcccttctccatcatcacactcttcaccggcagacgcattcctccggtacctactgaaaaaccagattcggccgaagaacgggccgggattctgtcaaaattgacctggcaatggcttagtccattgttgaaagtgagtatggctataggataacttctgatgtcttcttcaatactaacacagactggttacttacgaaacattgaacgtgaggatctgtataaagtgagagagagaaactcggcggctgtgatccagcagcgacttgaatccaatctcgaaaaacaatacgccaagtaccacgccaaactgctcaagaaaggactctcggagcaagaggcgcatctcaagctgcaagattcagccaaacccctcgtcttggctcttaaccagacgtttttttggaagttctggctagccggactgtttgccctagtcaaggacctctgtggaatcgcctcagctatggtgtcacgtgttctgatcgaatacattcaagacagatatctctacagggggacagaccgggaacctaaggtcggccgaggagtcggcccctcgataggcctatttctactggccgtaggagtcactttcttcttcaaccacatgttctacaatgtcaagatggttggagctcaggctcgtgcagctctggtggccgtcatctacagcaagagtacccgtttgagcgccaagggccgagctcaatacaccacaggcaagatcacaaacttggcagctattgacgcacatcgagttgatctcagttgtgaatctttccactacattactatctttttgcctgttgtgggttgtgccattgctgtactcgtggtcaacctcaaggtcgcagctctagttggaattgcgaccatgattgtcttgatctttgtcgtcgcaggcatcaccatcttctctatgaagctgcgagccatcattgtcaagctcacggataagcgagtcacgtatatccgagaagctctgcagtcgattagaatcatcaagtactacggctgggaggttccttactgtgacaagatcaagaaggtgcgtcttgacgagacccgtaactacgccaagatgggctcgattcgaggaacagccattggtatgtttcaggcactccctattttggcaggagcgttgtctttcatcacctacgctgctctaggtcatggaactgatcctgctcgaatgttctcttctctgacgcttttcaatttactcctgcctgctcttgctgttcttccccaggccctccaggctgctggagacgctcgagtggctctcagacgtatccagcggttccttggggccgaggagtcgactcccactacagtttttgacgctactcttgaatctactgatgacgctgtgattgtggaagacgcctctttcatctggccagaagttgtcgatgataagagcgacaaagagaaggctaaagatgcaaagaaggaggaaaaggataagaagaaggccgagaagaaggccaagaaggcggccaagaaggcggccaaggagatcgcggtggttgtggaagaggaggtggaacacgaaaagaccgagggatccagtgagtctgaaaagggtactcttaagtcgactttcaagggcttcaacaacctgtctttcaaaatcaagcggggtgaatttgtcgttgttaccggtcccattggttctggaaagtcgtctcttcttgctgccatcactggatctatggttttgacaggcggttccgtgcgagtgtcgtccacagagtggattggatgtctggagccgtggattcaaaacgccacagttcgagataacattgtgtttgggcgaaaattcgactctgaatggtatagaactgtggttactgcctgtcagctgagccaggatctcaaaataatgactcacggagacaataccatgattggagagcgaggcatcacagtttcgggcggtcaaaaagctcgaatcaacctcgcacgtgctatatatggaaaccccgagattctcatcatggacgacgtcctgtcggctgtggacgctcgagtaggtgctggtattgtggacgattgtcttcgaggcttagccaagaactccactcgaattctggccacccatcagctgtctgtgctgcctaaggctgatcatgtgattttcatggatgccgaaggccagtttcatattggtacgtaccaagagctggaggctgacaatgagcagttcaaggctcttttggcggctggttccatgtccaaggaggaggtggttgctgtcgacgagactgaggttgttattgaaggcgatcttgaagacgactgcgataacaaggaggagtatgaggatgcagctgagaccatttccattttggcagatgccactcaagagctgcaaaaggtgaccactacagtctcggcatttgaggagaacgataacatgatggaggaagaagagcgaatgagagatgcagttggtttgcatgtgtactggcagtattttcgtcaggccaaccccagtagggtcaaggtaatgatgttcattggcatgatcttcatttccatgattgtgattgcctttctgtttgtcttcacatctgtatggctctcgttctggacaggtgaccgtttccatgcctccagaaacttctacaccggaatttacatcatgctgggtattcttctgcttcttgctgtggcaggatacatgattgtcaatgagatcaactctgccatggcagcaagaaatctacacaatcatgctttggactcggtgttcgctgcacgaacttctttcttcgataccactcctcagggtcgtatcatcaaccggttcacccgagacacagactctctggataacgagctggctatgcgattgactatgttgttctttggcgtctccgcattcttctccaacttcctgcttacttgtgtctacgttccttatgtgactcttgtgcttgtccctgtcggttttgtcttctacgtttctctaggttactaccgaaagtcagctcgtgaagtcaagcgaattgactccattgaacggtcgcacatgatgagtgtcttcaacgagtccatttccggtatgcccgtcatcatcatgtacaaggcccagcatcggctcatgaacaagcttcaggctactctcgatgatatggacagtgcctacttcctcactgctgcaaaccagcgatggctgtctctccgtctggatggtctgggttctttggtcgttctggtggccactattcttgttgctgtcggagtctttgatctcaccccttccaacatgggtctgatcatttccgcggcctcctttatccccgaagtcatgtctatggttgcccaggccgttgctgaactcgaaaactgcatgaacgccacagagcgaattctttactacaaggacaacattcctgctgaggctgctcgagaagtggacggtacagagctcgaccagcgacccaactggcctgagcagggagccatcagcttcaacaatgtgtccatgaagtaccgagatggacttccttacgtgctcaagtcattgtctgtcgactttcagggaggacacaaggtgggtatctgtggacgaacaggagccggtaagagtaccatcttgcagactctgtatcgaattgtggagcttgctgagggttctattactattgatggtgttgacatttcgactattggactgcatcagcttcggtctcagttgtccatcattccccaggagccagttttgttcctgggcaccatccggtctaatttggatcctctggagcaatactctgatgctgagctatggggttctctacgacggtctggacttctcgatgaaggagagactgagggtaagtttcatctggatcaaaaggtggaggctgacggcagcaacttctctctaggtgagcgacagctgctgactctagcccgagcactgcttagaaacaccaaaattttggtgctggacgaagccacatcaaatgtcgactacaagacggacaagctggttcaggagaccatttcacgggagtttggccactgcacgattctgtgtatcgcccatcgactgcgaaccattgccaagtatgatcgtattttggtgcttgagtccggcgagatcaaccagtacgacacgccctggaacttgtacaacgacaaggagggtattttccgaggtatgtgtgacacctccgggttgaacgaggtagacttcaacaagtga

SEQ ID NO: 2 - DNA, 6595 bp, Yarrowia lipolytica
  misc_feature: Genomic sequence of the Yarrowia lipolytica transporter YALI0E25201 comprising a 1000 bp flanking sequence upstream of the ORF, the ORF and, downstream of the ORF, the terminator sequence (300 bp) followed by a 999 bp flanking sequence
cacaaagtacaatacaagtacatactgtacctgtgagtcatagtgacatgagaaaccatcgaaggggcacacactcactcacactgtgaattggctctggtcgactgcctgatgctcctataatcgatctacacaccaactcctttctcatccgcatggatatagtttcatatcagtgtgcatggtgcaaaacgccgtttgccacccaatagtgttctgtgcactaatttgacagcgaatttgccactgtggggaacgtggggaggaactggaactacggtactcgttcgaagttccgatccgaccggtgtgtgtcgagcaatggagtctgtgaaacctgtagtggtgctcgtggtggtggtggtggtggttgcacttgcagcatgtaagcagctgacgcgtcgcttaatagcacagtcagttcgtatactgtgatacttcaatggtgtcaggaaggtgaagaaacaacgggtaatagggcatgttccatttattttgaacttgctgcttgaagtaggtttggagactgcgttcggtgcattagcttcttgatatggaggcacggctcttcggggtccgaggtcgtggatagaagttggaaagaggttctcggggttcttgtagatgaaaaaaacgacgaagttgagataattaaacactgtggagaagagatatcgactgctgtgggtcacataacctcttatatacgcgccaattctttcaccaacccgcaagtccccaaactcaatccagaagactatcaattttagacatgtatcggtcacatcaatcgccgataaccaaccagcaagtggggagacgccacctttttctcgcagcttttatactcggcactgcggcgttgctacttaacctccttgaatctcgattggactgctagatcattgagatcagtcgacaaacagctcagatcagccacagatcagacagctgatttcagatcatcagtttctcacaccacaccctcagtcttccacacatgggtaaaaccgaagtgacacaggagagtctagaatgcgggtcggtcacgtcctcgctggggaaaaagcccttctccatcatcacactcttcaccggcagacgcattcctccggtacctactgaaaaaccagattcggccgaagaacgggccgggattctgtcaaaattgacctggcaatggcttagtccattgttgaaagtgagtatggctataggataacttctgatgtcttcttcaatactaacacagactggttacttacgaaacattgaacgtgaggatctgtataaagtgagagagagaaactcggcggctgtgatccagcagcgacttgaatccaatctcgaaaaacaatacgccaagtaccacgccaaactgctcaagaaaggactctcggagcaagaggcgcatctcaagctgcaagattcagccaaacccctcgtcttggctcttaaccagacgtttttttggaagttctggctagccggactgtttgccctagtcaaggacctctgtggaatcgcctcagctatggtgtcacgtgttctgatcgaatacattcaagacagatatctctacagggggacagaccgggaacctaaggtcggccgaggagtcggcccctcgataggcctatttctactggccgtaggagtcactttcttcttcaaccacatgttctacaatgtcaagatggttggagctcaggctcgtgcagctctggtggccgtcatctacagcaagagtacccgtttgagcgccaagggccgagctcaatacaccacaggcaagatcacaaacttggcagctattgacgcacatcgagttgatctcagttgtgaatctttccactacattactatctttttgcctgttgtgggttgtgccattgctgtactcgtggtcaacctcaaggtcgcagctctagttggaattgcgaccatgattgtcttgatctttgtcgtcgcaggcatcaccatcttctctatgaagctgcgagccatcattgtcaagctcacggataagcgagtcacgtatatccgagaagctctgcagtcgattagaatcatcaagtactacggctgggaggttccttactgtgacaagatcaagaaggtgcgtcttgacgagacccgtaactacgccaagatgggctcgattcgaggaacagccattggtatgtttcaggcactccctattttggcaggagcgttgtctttcatcacctacgctgctctaggtcatggaactgatcctgctcgaatgttctcttctctgacgcttttcaatttactcctgcctgctcttgctgttcttccccaggccctccaggctgctggagacgctcgagtggctctcagacgtatccagcggttccttggggccgaggagtcgactcccactacagtttttgacgctactcttgaatctactgatgacgctgtgattgtggaagacgcctctttcatctggccagaagttgtcgatgataagagcgacaaagagaaggctaaagatgcaaagaaggaggaaaaggataagaagaaggccgagaagaaggccaagaaggcggccaagaaggcggccaaggagatcgcggtggttgtggaagaggaggtggaacacgaaaagaccgagggatccagtgagtctgaaaagggtactcttaagtcgactttcaagggcttcaacaacctgtctttcaaaatcaagcggggtgaatttgtcgttgttaccggtcccattggttctggaaagtcgtctcttcttgctgccatcactggatctatggttttgacaggcggttccgtgcgagtgtcgtccacagagtggattggatgtctggagccgtggattcaaaacgccacagttcgagataacattgtgtttgggcgaaaattcgactctgaatggtatagaactgtggttactgcctgtcagctgagccaggatctcaaaataatgactcacggagacaataccatgattggagagcgaggcatcacagtttcgggcggtcaaaaagctcgaatcaacctcgcacgtgctatatatggaaaccccgagattctcatcatggacgacgtcctgtcggctgtggacgctcgagtaggtgctggtattgtggacgattgtcttcgaggcttagccaagaactccactcgaattctggccacccatcagctgtctgtgctgcctaaggctgatcatgtgattttcatggatgccgaaggccagtttcatattggtacgtaccaagagctggaggctgacaatgagcagttcaaggctcttttggcggctggttccatgtccaaggaggaggtggttgctgtcgacgagactgaggttgttattgaaggcgatcttgaagacgactgcgataacaaggaggagtatgaggatgcagctgagaccatttccattttggcagatgccactcaagagctgcaaaaggtgaccactacagtctcggcatttgaggagaacgataacatgatggaggaagaagagcgaatgagagatgcagttggtttgcatgtgtactggcagtattttcgtcaggccaaccccagtagggtcaaggtaatgatgttcattggcatgatcttcatttccatgattgtgattgcctttctgtttgtcttcacatctgtatggctctcgttctggacaggtgaccgtttccatgcctccagaaacttctacaccggaatttacatcatgctgggtattcttctgcttcttgctgtggcaggatacatgattgtcaatgagatcaactctgccatggcagcaagaaatctacacaatcatgctttggactcggtgttcgctgcacgaacttctttcttcgataccactcctcagggtcgtatcatcaaccggttcacccgagacacagactctctggataacgagctggctatgcgattgactatgttgttctttggcgtctccgcattcttctccaacttcctgcttacttgtgtctacgttccttatgtgactcttgtgcttgtccctgtcggttttgtcttctacgtttctctaggttactaccgaaagtcagctcgtgaagtcaagcgaattgactccattgaacggtcgcacatgatgagtgtcttcaacgagtccatttccggtatgcccgtcatcatcatgtacaaggcccagcatcggctcatgaacaagcttcaggctactctcgatgatatggacagtgcctacttcctcactgctgcaaaccagcgatggctgtctctccgtctggatggtctgggttctttggtcgttctggtggccactattcttgttgctgtcggagtctttgatctcaccccttccaacatgggtctgatcatttccgcggcctcctttatccccgaagtcatgtctatggttgcccaggccgttgctgaactcgaaaactgcatgaacgccacagagcgaattctttactacaaggacaacattcctgctgaggctgctcgagaagtggacggtacagagctcgaccagcgacccaactggcctgagcagggagccatcagcttcaacaatgtgtccatgaagtaccgagatggacttccttacgtgctcaagtcattgtctgtcgactttcagggaggacacaaggtgggtatctgtggacgaacaggagccggtaagagtaccatcttgcagactctgtatcgaattgtggagcttgctgagggttctattactattgatggtgttgacatttcgactattggactgcatcagcttcggtctcagttgtccatcattccccaggagccagttttgttcctgggcaccatccggtctaatttggatcctctggagcaatactctgatgctgagctatggggttctctacgacggtctggacttctcgatgaaggagagactgagggtaagtttcatctggatcaaaaggtggaggctgacggcagcaacttctctctaggtgagcgacagctgctgactctagcccgagcactgcttagaaacaccaaaattttggtgctggacgaagccacatcaaatgtcgactacaagacggacaagctggttcaggagaccatttcacgggagtttggccactgcacgattctgtgtatcgcccatcgactgcgaaccattgccaagtatgatcgtattttggtgcttgagtccggcgagatcaaccagtacgacacgccctggaacttgtacaacgacaaggagggtattttccgaggtatgtgtgacacctccgggttgaacgaggtagacttcaacaagtgaaaaattacgatgagggtagacagtctgagatgagactgataaattatagagaaaaaatgtttgattatagcagtagtgaatgtattgtatgtaataagtggccaatcttggaatggtggcctccgtattaattcttaccgaactcgtagtcacctttgtaaagcgacagtgtctgttcacattgggtcaaacatgtaaatattgtagctacgtagtctatagtcctaagagaacgataccatagaaaatcgatttccacagccgatcttttttgtcggtggcaatcagtacttttctttttctcaatattcgcaccgttcacaattacctcaaattgcttttcggaagttgagataggatcgggtcgggagtgtttcggaagcgggtcgggccgaaaaagccgttaccgggtttccgaaactgcctctgaaaagatgtggaatcacatgggggagtattagcagtgcctttgagatgtttcggttgagctctgcttagctttcattaggcaagagccgtgcttgatagatttctcgagcatgtagctcatactagctcttgcaccattgaggtgaggtgaatgaggtgctgtatccgtttttgatgacaccaattgataataattgtgagttatggcaacgcaaagagtttgttagaatgatagcagagaaattccatgcgaaacaccgctatatggcttgtttggcagagtcctacttcagctgtggtgttcatgccgaactatagtatgtacgagaacaaagtagcccattacaatcacaagcggtcgtcgatactcaatcaaaaataaacgtccagccaatgctacatcaaagacacccttcaaacagcatctggacccgcagacttgccactatggatgcaggacgttaaggggtggcatcaagccgcagagagactatacgagtcttggctaactgtaattaggtgacaattgagagtgatgtccactgataggctacttttacgagtgataagtgagagcgatagcctcggcgtctaaaaagggagcacaatgagtgtcttattacgagtacggtgatatacattgttgttcatctatagtttggatgtgtgtcaggtgcccgtttttatcagttcaccctacgagtacatacagtatgtacttgtacagtacacttacaagatctagtttgaccatgcaactgaacagaatacaactaaacagatttagttacacgcatacacacaatagggtgtataacctcagatatcagtcccatacttatagtactgtattgttgtccttcacattct

SEQ ID NO: 3 - protein, 1414 aa, Yarrowia lipolytica
  MISC_FEATURE: Amino acid sequence of the Yarrowia lipolytica transporter YALI0E25201
MGKTEVTQESLECGSVTSSLGKKPFSIITLFTGRRIPPVPTEKPDSAEERAGILSKLTWQWLSPLLKTGYLRNIEREDLYKVRERNSAAVIQQRLESNLEKQYAKYHAKLLKKGLSEQEAHLKLQDSAKPLVLALNQTFFWKFWLAGLFALVKDLCGIASAMVSRVLIEYIQDRYLYRGTDREPKVGRGVGPSIGLFLLAVGVTFFFNHMFYNVKMVGAQARAALVAVIYSKSTRLSAKGRAQYTTGKITNLAAIDAHRVDLSCESFHYITIFLPVVGCAIAVLVVNLKVAALVGIATMIVLIFVVAGITIFSMKLRAIIVKLTDKRVTYIREALQSIRIIKYYGWEVPYCDKIKKVRLDETRNYAKMGSIRGTAIGMFQALPILAGALSFITYAALGHGTDPARMFSSLTLFNLLLPALAVLPQALQAAGDARVALRRIQRFLGAEESTPTTVFDATLESTDDAVIVEDASFIWPEVVDDKSDKEKAKDAKKEEKDKKKAEKKAKKAAKKAAKEIAVVVEEEVEHEKTEGSSESEKGTLKSTFKGFNNLSFKIKRGEFVVVTGPIGSGKSSLLAAITGSMVLTGGSVRVSSTEWIGCLEPWIQNATVRDNIVFGRKFDSEWYRTVVTACQLSQDLKIMTHGDNTMIGERGITVSGGQKARINLARAIYGNPEILIMDDVLSAVDARVGAGIVDDCLRGLAKNSTRILATHQLSVLPKADHVIFMDAEGQFHIGTYQELEADNEQFKALLAAGSMSKEEVVAVDETEVVIEGDLEDDCDNKEEYEDAAETISILADATQELQKVTTTVSAFEENDNMMEEEERMRDAVGLHVYWQYFRQANPSRVKVMMFIGMIFISMIVIAFLFVFTSVWLSFWTGDRFHASRNFYTGIYIMLGILLLLAVAGYMIVNEINSAMAARNLHNHALDSVFAARTSFFDTTPQGRIINRFTRDTDSLDNELAMRLTMLFFGVSAFFSNFLLTCVYVPYVTLVLVPVGFVFYVSLGYYRKSAREVKRIDSIERSHMMSVFNESISGMPVIIMYKAQHRLMNKLQATLDDMDSAYFLTAANQRWLSLRLDGLGSLVVLVATILVAVGVFDLTPSNMGLIISAASFIPEVMSMVAQAVAELENCMNATERILYYKDNIPAEAAREVDGTELDQRPNWPEQGAISFNNVSMKYRDGLPYVLKSLSVDFQGGHKVGICGRTGAGKSTILQTLYRIVELAEGSITIDGVDISTIGLHQLRSQLSIIPQEPVLFLGTIRSNLDPLEQYSDAELWGSLRRSGLLDEGETEGKFHLDQKVEADGSNFSLGERQLLTLARALLRNTKILVLDEATSNVDYKTDKLVQETISREFGHCTILCIAHRLRTIAKYDRILVLESGEINQYDTPWNLYNDKEGIFRGMCDTSGLNEVDFNK

SEQ ID NO: 4 - protein, 500 aa, Artificial sequence
  Truncated 3-hydroxy-3-methylglutaryl coenzyme A reductase
MTQSVKVVEKHVPIVIEKPSEKEEDTSSEDSIELTVGKQPKPVTETRSLDDLEAIMKAGKTKLLEDHEVVKLSLEGKLPLYALEKQLGDNTRAVGIRRSIISQQSNTKTLETSKLPYLHYDYDRVFGACCENVIGYMPLPVGVAGPMNIDGKNYHIPMATTEGCLVASTMRGCKAINAGGGVTTVLTQDGMTRGPCVSFPSLKRAGAAKIWLDSEEGLKSMRKAFNSTSRFARLQSLHSTLAGNLLFIRFRTTTGDAMGMNMISKGVEHSLAVMVKEYGFPDMDIVSVSGNYCTDKKPAAINWIEGRGKSVVAEATIPAHIVKSVLKSEVDALVELNISKNLIGSAMAGSVGGFNAHAANLVTAIYLATGQDPAQNVESSNCITLMSNVDGNLLISVSMPSIEVGTIGGGTILEPQGAMLEMLGVRGPHIETPGANAQQLARIIASGVLAAELSLCSALAAGHLVQSHMTHNRSQAPTPAKQSQADLQRLQNGSNICIRS

SEQ ID NO: 5 - protein, 327 aa, Artificial sequence
  Variant geranylgeranyl-diphosphate synthase
MDYNSADFKEIWGKAADTALLGPYNYLANNRGHNIREHLIAAFGAVIKVDKSDLETISHITKILHNSSLLVDDVEDNSMLRRGLPAAHCLFEVPQTINSVNYMYFVALQEVLKLKSYDAVSIFTEEMINLHRGQGMDLYWRETLTCPSEDEYLEMVVHKTGGLFRLALRLMLSVASKQEDHEKINFDLTHLTDTLGVIYQILDDYLNLQSTELTENKGFCEDISEGKFSFPLIHSIRTNPDNHEILNILKQRTSDASLKKYAVDYMRTETKSFDYCLKRIQAMSLKASSYIDDLAAAGHDVSKLRAILHYFVSTSDCEERKYFEDAQ

SEQ ID NO: 6 - protein, 525 aa, Artificial sequence
  Variant kaurenoic acid 13-hydroxylase
MESLVVHTVNAIWCIVIVGIFSVGYHVYGRAVVEQWRMRRSLKLQGVKGPPPSIFNGNVSEMQRIQSEAKHNSGDNIISHDYSSTLFPHFDHWRKQYGRIYTYSTGLRQHLYINHPEMVKELSQTNSLDLGRITHVTKRLAPILGNGIITSNGPHWAHQRRIIAYEFTHDKVKGMVGLMVESAMPMLNKWEEMVEAEGGMGCDIRVDEDLKDVSADVIAKACFGSNFSKGKAIFSKIRDLLTAITKRSVLFRFNGFTDMVFGSKKHGDVDIDALEMELESSIWETVKERERECKDTHKKDLLQLILEGAMRSCDGNLWDKSAYRRFVVDNCKSIYFAGHDSTAVSVSWCLMLLALNPSWQEKIRDEILSSCKNGIPDAESIPNLKTVTMVIQETMRLYPPAPIVGREASKDIRLGDLVVPKGVCIWTLIPALHRDPEIWGPDANDFKPERFSEGISKACKYPQAYIPFGLGPRTCVGKNFGMMEVKVLVSLIVSKFSFTLSPTYQHSPSHKLLVEPQHGVVIRVV